European Patent Application EP 4 755 916 A1, published June 10, 2026. Title: BTN3A结合蛋白及其医药用途. Applicant: 江苏恒瑞医药股份有限公司. Application WO. The sequence listing filed with the application follows.

SEQUENCE LISTING (64 sequences)

SEQ ID NO: 1 - protein, 114 aa, Leporidae
QSLEESGGRLVTPGTPLTLTCTASGFSLNDYYITWVRQAPGKGLEWIGVIYGSSNTVYASWAKGRFTISKTSTMVDLRITSPTTEDTATYFCARGYLASSADIWGPGTLVTVSL

SEQ ID NO: 2 - protein, 109 aa, Leporidae
QVLTQTPSPVSAAVGGTVTINCQSSQSVYNNNRLAWYQQKPGQPPKLLIYDASTLASGVPSRFKGSGSGTDFTLTISDLECADAATYYCQTYYSGYIWAFGGGTEVVVK

SEQ ID NO: 3 - protein, 116 aa, Leporidae
QSVEESGGRLVTPGTPLTLTCTASGFTINNYYMNWVRQAPGKGLEWIGIIYGSDNTYYASWAKGRFTISKTSTTVDLIMTSPTTEDTATYFCVRNLDYSSAYFHIWGPGTLVTVSS

SEQ ID NO: 4 - protein, 109 aa, Leporidae
QVLTQTPSPVSAAVGGTVSISCQASQSVYNNNRLAWYQQKPGQPPNLLIYEASKLASGVPSRFKGSGSGTQFTLIISEVQCEDAATYYCQGYYSGFIYPFGGGTEVVVK

SEQ ID NO: 5 - protein, 5 aa, Leporidae
DYYIT

SEQ ID NO: 6 - protein, 16 aa, Leporidae
VIYGSSNTVYASWAKG

SEQ ID NO: 7 - protein, 9 aa, Leporidae
GYLASSADI

SEQ ID NO: 8 - protein, 13 aa, Leporidae
QSSQSVYNNNRLA

SEQ ID NO: 9 - protein, 7 aa, Leporidae
DASTLAS

SEQ ID NO: 10 - protein, 10 aa, Leporidae
QTYYSGYIWA

SEQ ID NO: 11 - protein, 5 aa, Leporidae
NYYMN

SEQ ID NO: 12 - protein, 16 aa, Leporidae
IIYGSDNTYYASWAKG

SEQ ID NO: 13 - protein, 11 aa, Leporidae
NLDYSSAYFHI

SEQ ID NO: 14 - protein, 13 aa, Leporidae
QASQSVYNNNRLA

SEQ ID NO: 15 - protein, 7 aa, Leporidae
EASKLAS

SEQ ID NO: 16 - protein, 10 aa, Leporidae
QGYYSGFIYP

SEQ ID NO: 17 - skipped

SEQ ID NO: 18 - protein, 16 aa, Artificial Sequence
  VARIANT 1: note = X is V or I
  VARIANT 6: note = X5 is S or D
  VARIANT 9: note = X is Vor Y
XIYGSXNTXYASWAKG

SEQ ID NO: 19 - skipped

SEQ ID NO: 20 - protein, 13 aa, Artificial Sequence
  VARIANT 2: note = X is S or A
QXSQSVYNNNRLA

SEQ ID NO: 21 - protein, 7 aa, Artificial Sequence
  VARIANT 1: note = X is D or E
  VARIANT 4: note = X is T or K
XASXLAS

SEQ ID NO: 22 - protein, 10 aa, Artificial Sequence
  VARIANT 2: note = X is T or G
  VARIANT 7: note = X is Y or F
  VARIANT 9: note = X is W or Y
  VARIANT 10: note = X is A or P
QXYYSGXIXX

SEQ ID NO: 23 - protein, 330 aa, Artificial Sequence
  source 1..330: note = Fc
ASTKGPSVFPLAPSSKSTSGGTAALGCLVKDYFPEPVTVSWNSGALTSGVHTFPAVLQSSGLYSLSSVVTVPSSSLGTQTYICNVNHKPSNTKVDKRVEPKSCDKTHTCPPCPAPEFEGGPSVFLFPPKPKDTLMISRTPEVTCVVVDVSHEDPEVKFNWYVDGVEVHNAKTKPREEQYNSTYRVVSVLTVLHQDWLNGKEYKCKVSNKALPASIEKTISKAKGQPREPQVYTLPPSREEMTKNQVSLTCLVKGFYPSDIAVEWESNGQPENNYKTTPPVLDSDGSFFLYSKLTVDKSRWQQGNVFSCSVMHEALHNHYTQKSLSLSPGK

SEQ ID NO: 24 - protein, 329 aa, Artificial Sequence
  source 1..329: note = Fc
ASTKGPSVFPLAPSSKSTSGGTAALGCLVKDYFPEPVTVSWNSGALTSGVHTFPAVLQSSGLYSLSSVVTVPSSSLGTQTYICNVNHKPSNTKVDKRVEPKSCDKTHTCPPCPAPEFEGGPSVFLFPPKPKDTLMISRTPEVTCVVVDVSHEDPEVKFNWYVDGVEVHNAKTKPREEQYNSTYRVVSVLTVLHQDWLNGKEYKCKVSNKALPASIEKTISKAKGQPREPQVYTLPPSREEMTKNQVSLTCLVKGFYPSDIAVEWESNGQPENNYKTTPPVLDSDGSFFLYSKLTVDKSRWQQGNVFSCSVMHEALHNHYTQKSLSLSPG

SEQ ID NO: 25 - protein, 444 aa, Artificial Sequence
  source 1..444: note = HC
QSLEESGGRLVTPGTPLTLTCTASGFSLNDYYITWVRQAPGKGLEWIGVIYGSSNTVYASWAKGRFTISKTSTMVDLRITSPTTEDTATYFCARGYLASSADIWGPGTLVTVSLASTKGPSVFPLAPSSKSTSGGTAALGCLVKDYFPEPVTVSWNSGALTSGVHTFPAVLQSSGLYSLSSVVTVPSSSLGTQTYICNVNHKPSNTKVDKRVEPKSCDKTHTCPPCPAPEFEGGPSVFLFPPKPKDTLMISRTPEVTCVVVDVSHEDPEVKFNWYVDGVEVHNAKTKPREEQYNSTYRVVSVLTVLHQDWLNGKEYKCKVSNKALPASIEKTISKAKGQPREPQVYTLPPSREEMTKNQVSLTCLVKGFYPSDIAVEWESNGQPENNYKTTPPVLDSDGSFFLYSKLTVDKSRWQQGNVFSCSVMHEALHNHYTQKSLSLSPGK

SEQ ID NO: 26 - protein, 216 aa, Artificial Sequence
  source 1..216: note = LC
QVLTQTPSPVSAAVGGTVTINCQSSQSVYNNNRLAWYQQKPGQPPKLLIYDASTLASGVPSRFKGSGSGTDFTLTISDLECADAATYYCQTYYSGYIWAFGGGTEVVVKRTVAAPSVFIFPPSDEQLKSGTASVVCLLNNFYPREAKVQWKVDNALQSGNSQESVTEQDSKDSTYSLSSTLTLSKADYEKHKVYACEVTHQGLSSPVTKSFNRGEC

SEQ ID NO: 27 - protein, 446 aa, Artificial Sequence
  source 1..446: note = HC
QSVEESGGRLVTPGTPLTLTCTASGFTINNYYMNWVRQAPGKGLEWIGIIYGSDNTYYASWAKGRFTISKTSTTVDLIMTSPTTEDTATYFCVRNLDYSSAYFHIWGPGTLVTVSSASTKGPSVFPLAPSSKSTSGGTAALGCLVKDYFPEPVTVSWNSGALTSGVHTFPAVLQSSGLYSLSSVVTVPSSSLGTQTYICNVNHKPSNTKVDKRVEPKSCDKTHTCPPCPAPEFEGGPSVFLFPPKPKDTLMISRTPEVTCVVVDVSHEDPEVKFNWYVDGVEVHNAKTKPREEQYNSTYRVVSVLTVLHQDWLNGKEYKCKVSNKALPASIEKTISKAKGQPREPQVYTLPPSREEMTKNQVSLTCLVKGFYPSDIAVEWESNGQPENNYKTTPPVLDSDGSFFLYSKLTVDKSRWQQGNVFSCSVMHEALHNHYTQKSLSLSPGK

SEQ ID NO: 28 - protein, 216 aa, Artificial Sequence
  source 1..216: note = LC
QVLTQTPSPVSAAVGGTVSISCQASQSVYNNNRLAWYQQKPGQPPNLLIYEASKLASGVPSRFKGSGSGTQFTLIISEVQCEDAATYYCQGYYSGFIYPFGGGTEVVVKRTVAAPSVFIFPPSDEQLKSGTASVVCLLNNFYPREAKVQWKVDNALQSGNSQESVTEQDSKDSTYSLSSTLTLSKADYEKHKVYACEVTHQGLSSPVTKSFNRGEC

SEQ ID NO: 29 - protein, 451 aa, Artificial Sequence
  source 1..451: note = HC
QVQLVQSGAEVKKPGASVKLSCKASGYIFTRYYMYWVKQRPGQGLEWIGEINPNNGGTKFNEKFKNRATLTVDKSISTAYMELSRLRSDDTAVYYCSREDDYDGTPFAMDYWGQGTLVTVSSASTKGPSVFPLAPSSKSTSGGTAALGCLVKDYFPEPVTVSWNSGALTSGVHTFPAVLQSSGLYSLSSVVTVPSSSLGTQTYICNVNHKPSNTKVDKRVEPKSCDKTHTCPPCPAPEFEGGPSVFLFPPKPKDTLMISRTPEVTCVVVDVSHEDPEVKFNWYVDGVEVHNAKTKPREEQYNSTYRVVSVLTVLHQDWLNGKEYKCKVSNKALPASIEKTISKAKGQPREPQVYTLPPSREEMTKNQVSLTCLVKGFYPSDIAVEWESNGQPENNYKTTPPVLDSDGSFFLYSKLTVDKSRWQQGNVFSCSVMHEALHNHYTQKSLSLSPG

SEQ ID NO: 30 - protein, 214 aa, Artificial Sequence
  source 1..214: note = LC
DIQMTQSPSSLSASVGDRVTITCHASQNINVWLSWYQQKPGKAPKLLIYKASNLHTGVPSRFTGSGSGTDFTFTISSLQPEDIATYYCQQGQTYPYTFGQGTKLEIKRTVAAPSVFIFPPSDEQLKSGTASVVCLLNNFYPREAKVQWKVDNALQSGNSQESVTEQDSKDSTYSLSSTLTLSKADYEKHKVYACEVTHQGLSSPVTKSFNRGEC

SEQ ID NO: 31 - protein, 117 aa, Artificial Sequence
  source 1..117: note = VH
EVQLVESGGGLVQPGGSLRLSCAASGFSLNDYYITWVRQAPGKGLEWVSVIYGSSNTVYASWAKGRFTISKDNSKNTVYLQMNSLRAEDTAVYYCARGYLASSADIWGQGTLVTVSS

SEQ ID NO: 32 - protein, 117 aa, Artificial Sequence
  source 1..117: note = VH
EVQLVESGGGLVQPGGSLRLSCAASGFSLNDYYITWVRQAPGKGLEWVSVIYGSSNTVYASWAKGRFTISKDNSKTTVYLQMNSLRAEDTAVYFCARGYLASSADIWGQGTLVTVSS

SEQ ID NO: 33 - protein, 117 aa, Artificial Sequence
  source 1..117: note = VH
EQQLVESGGGLVQPGGSLRLSCAASGFSLNDYYITWVRQAPGKGLEWVSVIYGSSNTVYASWAKGRFTISKDNSKTTVYLQMNSLRAEDTAVYFCARGYLASSADIWGQGTLVTVSS

SEQ ID NO: 34 - protein, 117 aa, Artificial Sequence
  source 1..117: note = VH
EQQLVESGGGLVQPGGSLRLSCAASGFSLNDYYITWVRQAPGKGLEWIGVIYGSSNTVYASWAKGRFTISKDNSKTTVYLQMNSLRAEDTAVYFCARGYLASSADIWGQGTLVTVSS

SEQ ID NO: 35 - protein, 115 aa, Artificial Sequence
  source 1..115: note = VH
EQQLVESGGGLVQPGGSLRLSCAASGFSLNDYYITWVRQAPGKGLEWIGVIYGSSNTVYASWAKGRFTISKTSTMVYLQMNSLRAEDTAVYFCARGYLASSADIWGQGTLVTVSS

SEQ ID NO: 36 - protein, 110 aa, Artificial Sequence
  source 1..110: note = VL
DIQLTQSPSSLSASVGDRVTITCQSSQSVYNNNRLAWYQQKPGKVPKLLIYDASTLASGVPSRFSGSGSGTDFTLTISSLQPEDVATYYCQTYYSGYIWAFGGGTKVEIK

SEQ ID NO: 37 - protein, 110 aa, Artificial Sequence
  source 1..110: note = VL
DIQLTQSPSSLSASVGDRVTITCQSSQSVYNNNRLAWYQQKPGKPPKLLIYDASTLASGVPSRFSGSGSGTDFTLTISSLQPEDVATYYCQTYYSGYIWAFGGGTKVEIK

SEQ ID NO: 38 - protein, 110 aa, Artificial Sequence
  source 1..110: note = VL
DQQLTQSPSSLSASVGDRVTITCQSSQSVYNNNRLAWYQQKPGKPPKLLIYDASTLASGVPSRFSGSGSGTDFTLTISSLQPEDVATYYCQTYYSGYIWAFGGGTKVEIK

SEQ ID NO: 39 - protein, 119 aa, Artificial Sequence
  source 1..119: note = VH
EVQLVESGGGLVQPGGSLRLSCAASGFTINNYYMNWVRQAPGKGLEWVSIIYGSDNTYYASWAKGRFTISRDNSKNTLYLQMNSLRAEDTAVYYCVRNLDYSSAYFHIWGQGTLVTVSS

SEQ ID NO: 40 - protein, 119 aa, Artificial Sequence
  source 1..119: note = VH
EVQLVESGGGLVQPGGSLRLSCAASGFTINNYYMNWVRQAPGKGLEWVSIIYGSDNTYYASWAKGRFTISKDNSKNTVYLQMNSLRAEDTAVYYCVRNLDYSSAYFHIWGQGTLVTVSS

SEQ ID NO: 41 - protein, 119 aa, Artificial Sequence
  source 1..119: note = VH
EVQVVESGGGLVQPGGSLRLSCAASGFTINNYYMNWVRQAPGKGLEWVSIIYGSDNTYYASWAKGRFTISKDNSKTTVYLQMNSLRAEDTAVYFCVRNLDYSSAYFHIWGQGTLVTVSS

SEQ ID NO: 42 - protein, 119 aa, Artificial Sequence
  source 1..119: note = VH
EQQVVESGGGLVQPGGSLRLSCAASGFTINNYYMNWVRQAPGKGLEWVSIIYGSDNTYYASWAKGRFTISKDNSKTTVYLQMNSLRAEDTAVYFCVRNLDYSSAYFHIWGQGTLVTVSS

SEQ ID NO: 43 - protein, 119 aa, Artificial Sequence
  source 1..119: note = VH
EQQVVESGGGLVQPGGSLRLSCAASGFTINNYYMNWVRQAPGKGLEWIGIIYGSDNTYYASWAKGRFTISKDNSKTTVYLQMNSLRAEDTAVYFCVRNLDYSSAYFHIWGQGTLVTVSS

SEQ ID NO: 44 - protein, 117 aa, Artificial Sequence
  source 1..117: note = VH
EQQVVESGGGLVQPGGSLRLSCAASGFTINNYYMNWVRQAPGKGLEWIGIIYGSDNTYYASWAKGRFTISKTSTTVYLQMNSLRAEDTAVYFCVRNLDYSSAYFHIWGQGTLVTVSS

SEQ ID NO: 45 - protein, 110 aa, Artificial Sequence
  source 1..110: note = VL
DIQLTQSPSSLSASVGDRVTITCQASQSVYNNNRLAWYQQKPGKVPKLLIYEASKLASGVPSRFSGSGSGTDFTLTISSLQPEDVATYYCQGYYSGFIYPFGGGTKVEIK

SEQ ID NO: 46 - protein, 110 aa, Artificial Sequence
  source 1..110: note = VL
DIQLTQSPSSLSASVGDRVTITCQASQSVYNNNRLAWYQQKPGKPPKLLIYEASKLASGVPSRFSGSGSGTDFTLTISSLQPEDVATYYCQGYYSGFIYPFGGGTKVEIK

SEQ ID NO: 47 - protein, 110 aa, Artificial Sequence
  source 1..110: note = VL
DQQLTQSPSSLSASVGDRVTITCQASQSVYNNNRLAWYQQKPGKPPKLLIYEASKLASGVPSRFSGSGSGTDFTLTISSLQPEDVATYYCQGYYSGFIYPFGGGTKVEIK

SEQ ID NO: 48 - protein, 447 aa, Artificial Sequence
  source 1..447: note = HC
EVQLVESGGGLVQPGGSLRLSCAASGFSLNDYYITWVRQAPGKGLEWVSVIYGSSNTVYASWAKGRFTISKDNSKNTVYLQMNSLRAEDTAVYYCARGYLASSADIWGQGTLVTVSSASTKGPSVFPLAPSSKSTSGGTAALGCLVKDYFPEPVTVSWNSGALTSGVHTFPAVLQSSGLYSLSSVVTVPSSSLGTQTYICNVNHKPSNTKVDKRVEPKSCDKTHTCPPCPAPEFEGGPSVFLFPPKPKDTLMISRTPEVTCVVVDVSHEDPEVKFNWYVDGVEVHNAKTKPREEQYNSTYRVVSVLTVLHQDWLNGKEYKCKVSNKALPASIEKTISKAKGQPREPQVYTLPPSREEMTKNQVSLTCLVKGFYPSDIAVEWESNGQPENNYKTTPPVLDSDGSFFLYSKLTVDKSRWQQGNVFSCSVMHEALHNHYTQKSLSLSPGK

SEQ ID NO: 49 - protein, 447 aa, Artificial Sequence
  source 1..447: note = HC
EVQLVESGGGLVQPGGSLRLSCAASGFSLNDYYITWVRQAPGKGLEWVSVIYGSSNTVYASWAKGRFTISKDNSKTTVYLQMNSLRAEDTAVYFCARGYLASSADIWGQGTLVTVSSASTKGPSVFPLAPSSKSTSGGTAALGCLVKDYFPEPVTVSWNSGALTSGVHTFPAVLQSSGLYSLSSVVTVPSSSLGTQTYICNVNHKPSNTKVDKRVEPKSCDKTHTCPPCPAPEFEGGPSVFLFPPKPKDTLMISRTPEVTCVVVDVSHEDPEVKFNWYVDGVEVHNAKTKPREEQYNSTYRVVSVLTVLHQDWLNGKEYKCKVSNKALPASIEKTISKAKGQPREPQVYTLPPSREEMTKNQVSLTCLVKGFYPSDIAVEWESNGQPENNYKTTPPVLDSDGSFFLYSKLTVDKSRWQQGNVFSCSVMHEALHNHYTQKSLSLSPGK

SEQ ID NO: 50 - protein, 447 aa, Artificial Sequence
  source 1..447: note = HC
EQQLVESGGGLVQPGGSLRLSCAASGFSLNDYYITWVRQAPGKGLEWVSVIYGSSNTVYASWAKGRFTISKDNSKTTVYLQMNSLRAEDTAVYFCARGYLASSADIWGQGTLVTVSSASTKGPSVFPLAPSSKSTSGGTAALGCLVKDYFPEPVTVSWNSGALTSGVHTFPAVLQSSGLYSLSSVVTVPSSSLGTQTYICNVNHKPSNTKVDKRVEPKSCDKTHTCPPCPAPEFEGGPSVFLFPPKPKDTLMISRTPEVTCVVVDVSHEDPEVKFNWYVDGVEVHNAKTKPREEQYNSTYRVVSVLTVLHQDWLNGKEYKCKVSNKALPASIEKTISKAKGQPREPQVYTLPPSREEMTKNQVSLTCLVKGFYPSDIAVEWESNGQPENNYKTTPPVLDSDGSFFLYSKLTVDKSRWQQGNVFSCSVMHEALHNHYTQKSLSLSPGK

SEQ ID NO: 51 - protein, 447 aa, Artificial Sequence
  source 1..447: note = HC
EQQLVESGGGLVQPGGSLRLSCAASGFSLNDYYITWVRQAPGKGLEWIGVIYGSSNTVYASWAKGRFTISKDNSKTTVYLQMNSLRAEDTAVYFCARGYLASSADIWGQGTLVTVSSASTKGPSVFPLAPSSKSTSGGTAALGCLVKDYFPEPVTVSWNSGALTSGVHTFPAVLQSSGLYSLSSVVTVPSSSLGTQTYICNVNHKPSNTKVDKRVEPKSCDKTHTCPPCPAPEFEGGPSVFLFPPKPKDTLMISRTPEVTCVVVDVSHEDPEVKFNWYVDGVEVHNAKTKPREEQYNSTYRVVSVLTVLHQDWLNGKEYKCKVSNKALPASIEKTISKAKGQPREPQVYTLPPSREEMTKNQVSLTCLVKGFYPSDIAVEWESNGQPENNYKTTPPVLDSDGSFFLYSKLTVDKSRWQQGNVFSCSVMHEALHNHYTQKSLSLSPGK

SEQ ID NO: 52 - protein, 445 aa, Artificial Sequence
  source 1..445: note = HC
EQQLVESGGGLVQPGGSLRLSCAASGFSLNDYYITWVRQAPGKGLEWIGVIYGSSNTVYASWAKGRFTISKTSTMVYLQMNSLRAEDTAVYFCARGYLASSADIWGQGTLVTVSSASTKGPSVFPLAPSSKSTSGGTAALGCLVKDYFPEPVTVSWNSGALTSGVHTFPAVLQSSGLYSLSSVVTVPSSSLGTQTYICNVNHKPSNTKVDKRVEPKSCDKTHTCPPCPAPEFEGGPSVFLFPPKPKDTLMISRTPEVTCVVVDVSHEDPEVKFNWYVDGVEVHNAKTKPREEQYNSTYRVVSVLTVLHQDWLNGKEYKCKVSNKALPASIEKTISKAKGQPREPQVYTLPPSREEMTKNQVSLTCLVKGFYPSDIAVEWESNGQPENNYKTTPPVLDSDGSFFLYSKLTVDKSRWQQGNVFSCSVMHEALHNHYTQKSLSLSPGK

SEQ ID NO: 53 - protein, 217 aa, Artificial Sequence
  source 1..217: note = LC
DIQLTQSPSSLSASVGDRVTITCQSSQSVYNNNRLAWYQQKPGKVPKLLIYDASTLASGVPSRFSGSGSGTDFTLTISSLQPEDVATYYCQTYYSGYIWAFGGGTKVEIKRTVAAPSVFIFPPSDEQLKSGTASVVCLLNNFYPREAKVQWKVDNALQSGNSQESVTEQDSKDSTYSLSSTLTLSKADYEKHKVYACEVTHQGLSSPVTKSFNRGEC

SEQ ID NO: 54 - protein, 217 aa, Artificial Sequence
  source 1..217: note = LC
DIQLTQSPSSLSASVGDRVTITCQSSQSVYNNNRLAWYQQKPGKPPKLLIYDASTLASGVPSRFSGSGSGTDFTLTISSLQPEDVATYYCQTYYSGYIWAFGGGTKVEIKRTVAAPSVFIFPPSDEQLKSGTASVVCLLNNFYPREAKVQWKVDNALQSGNSQESVTEQDSKDSTYSLSSTLTLSKADYEKHKVYACEVTHQGLSSPVTKSFNRGEC

SEQ ID NO: 55 - protein, 217 aa, Artificial Sequence
  source 1..217: note = LC
DQQLTQSPSSLSASVGDRVTITCQSSQSVYNNNRLAWYQQKPGKPPKLLIYDASTLASGVPSRFSGSGSGTDFTLTISSLQPEDVATYYCQTYYSGYIWAFGGGTKVEIKRTVAAPSVFIFPPSDEQLKSGTASVVCLLNNFYPREAKVQWKVDNALQSGNSQESVTEQDSKDSTYSLSSTLTLSKADYEKHKVYACEVTHQGLSSPVTKSFNRGEC

SEQ ID NO: 56 - protein, 449 aa, Artificial Sequence
  source 1..449: note = HC
EVQLVESGGGLVQPGGSLRLSCAASGFTINNYYMNWVRQAPGKGLEWVSIIYGSDNTYYASWAKGRFTISRDNSKNTLYLQMNSLRAEDTAVYYCVRNLDYSSAYFHIWGQGTLVTVSSASTKGPSVFPLAPSSKSTSGGTAALGCLVKDYFPEPVTVSWNSGALTSGVHTFPAVLQSSGLYSLSSVVTVPSSSLGTQTYICNVNHKPSNTKVDKRVEPKSCDKTHTCPPCPAPEFEGGPSVFLFPPKPKDTLMISRTPEVTCVVVDVSHEDPEVKFNWYVDGVEVHNAKTKPREEQYNSTYRVVSVLTVLHQDWLNGKEYKCKVSNKALPASIEKTISKAKGQPREPQVYTLPPSREEMTKNQVSLTCLVKGFYPSDIAVEWESNGQPENNYKTTPPVLDSDGSFFLYSKLTVDKSRWQQGNVFSCSVMHEALHNHYTQKSLSLSPGK

SEQ ID NO: 57 - protein, 449 aa, Artificial Sequence
  source 1..449: note = HC
EVQLVESGGGLVQPGGSLRLSCAASGFTINNYYMNWVRQAPGKGLEWVSIIYGSDNTYYASWAKGRFTISKDNSKNTVYLQMNSLRAEDTAVYYCVRNLDYSSAYFHIWGQGTLVTVSSASTKGPSVFPLAPSSKSTSGGTAALGCLVKDYFPEPVTVSWNSGALTSGVHTFPAVLQSSGLYSLSSVVTVPSSSLGTQTYICNVNHKPSNTKVDKRVEPKSCDKTHTCPPCPAPEFEGGPSVFLFPPKPKDTLMISRTPEVTCVVVDVSHEDPEVKFNWYVDGVEVHNAKTKPREEQYNSTYRVVSVLTVLHQDWLNGKEYKCKVSNKALPASIEKTISKAKGQPREPQVYTLPPSREEMTKNQVSLTCLVKGFYPSDIAVEWESNGQPENNYKTTPPVLDSDGSFFLYSKLTVDKSRWQQGNVFSCSVMHEALHNHYTQKSLSLSPGK

SEQ ID NO: 58 - protein, 449 aa, Artificial Sequence
  source 1..449: note = HC
EVQVVESGGGLVQPGGSLRLSCAASGFTINNYYMNWVRQAPGKGLEWVSIIYGSDNTYYASWAKGRFTISKDNSKTTVYLQMNSLRAEDTAVYFCVRNLDYSSAYFHIWGQGTLVTVSSASTKGPSVFPLAPSSKSTSGGTAALGCLVKDYFPEPVTVSWNSGALTSGVHTFPAVLQSSGLYSLSSVVTVPSSSLGTQTYICNVNHKPSNTKVDKRVEPKSCDKTHTCPPCPAPEFEGGPSVFLFPPKPKDTLMISRTPEVTCVVVDVSHEDPEVKFNWYVDGVEVHNAKTKPREEQYNSTYRVVSVLTVLHQDWLNGKEYKCKVSNKALPASIEKTISKAKGQPREPQVYTLPPSREEMTKNQVSLTCLVKGFYPSDIAVEWESNGQPENNYKTTPPVLDSDGSFFLYSKLTVDKSRWQQGNVFSCSVMHEALHNHYTQKSLSLSPGK

SEQ ID NO: 59 - protein, 449 aa, Artificial Sequence
  source 1..449: note = HC
EQQVVESGGGLVQPGGSLRLSCAASGFTINNYYMNWVRQAPGKGLEWVSIIYGSDNTYYASWAKGRFTISKDNSKTTVYLQMNSLRAEDTAVYFCVRNLDYSSAYFHIWGQGTLVTVSSASTKGPSVFPLAPSSKSTSGGTAALGCLVKDYFPEPVTVSWNSGALTSGVHTFPAVLQSSGLYSLSSVVTVPSSSLGTQTYICNVNHKPSNTKVDKRVEPKSCDKTHTCPPCPAPEFEGGPSVFLFPPKPKDTLMISRTPEVTCVVVDVSHEDPEVKFNWYVDGVEVHNAKTKPREEQYNSTYRVVSVLTVLHQDWLNGKEYKCKVSNKALPASIEKTISKAKGQPREPQVYTLPPSREEMTKNQVSLTCLVKGFYPSDIAVEWESNGQPENNYKTTPPVLDSDGSFFLYSKLTVDKSRWQQGNVFSCSVMHEALHNHYTQKSLSLSPGK

SEQ ID NO: 60 - protein, 449 aa, Artificial Sequence
  source 1..449: note = HC
EQQVVESGGGLVQPGGSLRLSCAASGFTINNYYMNWVRQAPGKGLEWIGIIYGSDNTYYASWAKGRFTISKDNSKTTVYLQMNSLRAEDTAVYFCVRNLDYSSAYFHIWGQGTLVTVSSASTKGPSVFPLAPSSKSTSGGTAALGCLVKDYFPEPVTVSWNSGALTSGVHTFPAVLQSSGLYSLSSVVTVPSSSLGTQTYICNVNHKPSNTKVDKRVEPKSCDKTHTCPPCPAPEFEGGPSVFLFPPKPKDTLMISRTPEVTCVVVDVSHEDPEVKFNWYVDGVEVHNAKTKPREEQYNSTYRVVSVLTVLHQDWLNGKEYKCKVSNKALPASIEKTISKAKGQPREPQVYTLPPSREEMTKNQVSLTCLVKGFYPSDIAVEWESNGQPENNYKTTPPVLDSDGSFFLYSKLTVDKSRWQQGNVFSCSVMHEALHNHYTQKSLSLSPGK

SEQ ID NO: 61 - protein, 447 aa, Artificial Sequence
  source 1..447: note = HC
EQQVVESGGGLVQPGGSLRLSCAASGFTINNYYMNWVRQAPGKGLEWIGIIYGSDNTYYASWAKGRFTISKTSTTVYLQMNSLRAEDTAVYFCVRNLDYSSAYFHIWGQGTLVTVSSASTKGPSVFPLAPSSKSTSGGTAALGCLVKDYFPEPVTVSWNSGALTSGVHTFPAVLQSSGLYSLSSVVTVPSSSLGTQTYICNVNHKPSNTKVDKRVEPKSCDKTHTCPPCPAPEFEGGPSVFLFPPKPKDTLMISRTPEVTCVVVDVSHEDPEVKFNWYVDGVEVHNAKTKPREEQYNSTYRVVSVLTVLHQDWLNGKEYKCKVSNKALPASIEKTISKAKGQPREPQVYTLPPSREEMTKNQVSLTCLVKGFYPSDIAVEWESNGQPENNYKTTPPVLDSDGSFFLYSKLTVDKSRWQQGNVFSCSVMHEALHNHYTQKSLSLSPGK

SEQ ID NO: 62 - protein, 217 aa, Artificial Sequence
  source 1..217: note = LC
DIQLTQSPSSLSASVGDRVTITCQASQSVYNNNRLAWYQQKPGKVPKLLIYEASKLASGVPSRFSGSGSGTDFTLTISSLQPEDVATYYCQGYYSGFIYPFGGGTKVEIKRTVAAPSVFIFPPSDEQLKSGTASVVCLLNNFYPREAKVQWKVDNALQSGNSQESVTEQDSKDSTYSLSSTLTLSKADYEKHKVYACEVTHQGLSSPVTKSFNRGEC

SEQ ID NO: 63 - protein, 217 aa, Artificial Sequence
  source 1..217: note = LC
DIQLTQSPSSLSASVGDRVTITCQASQSVYNNNRLAWYQQKPGKPPKLLIYEASKLASGVPSRFSGSGSGTDFTLTISSLQPEDVATYYCQGYYSGFIYPFGGGTKVEIKRTVAAPSVFIFPPSDEQLKSGTASVVCLLNNFYPREAKVQWKVDNALQSGNSQESVTEQDSKDSTYSLSSTLTLSKADYEKHKVYACEVTHQGLSSPVTKSFNRGEC

SEQ ID NO: 64 - protein, 217 aa, Artificial Sequence
  source 1..217: note = LC
DQQLTQSPSSLSASVGDRVTITCQASQSVYNNNRLAWYQQKPGKPPKLLIYEASKLASGVPSRFSGSGSGTDFTLTISSLQPEDVATYYCQGYYSGFIYPFGGGTKVEIKRTVAAPSVFIFPPSDEQLKSGTASVVCLLNNFYPREAKVQWKVDNALQSGNSQESVTEQDSKDSTYSLSSTLTLSKADYEKHKVYACEVTHQGLSSPVTKSFNRGEC